European Patent Specification EP 4 050 099 B1, published June 26, 2024. Title: Novel Peptide methionine sulfoxide reductase variant and a method for producing IMP using the same. Applicant: CJ CheilJedang Corporation. The sequence listing filed with the application follows.

SEQUENCE LISTING (11 sequences)

SEQ ID NO: 1 - protein, 216 aa, Artificial Sequence
  variant AA
MSFLFVPTPQLVAKEDALPGRAEPILEPKPHAVLGTPITGPWKEGQRSLLVALGCFWGHEKMYWETDGVESTSVGYAGGTTPNPTYFEVCRGQTNHAEVVEITYDPEKISLKELVVMALEAHDPTQGFRQGNDVGTQYRSAFYPRTQEELEIIQELVDSYDKKLAENGFGAMTTEVKLLSDTDSGEYYLAEDEHQQYLYKVPNGYCPHHSTGVKCD

SEQ ID NO: 2 - DNA, 651 bp, Artificial Sequence
  variant NT
atgtcgttcttatttgtacctacccctcaacttgttgctaaagaagatgcattacccggccgcgcagaacctatcttggagcctaagccgcatgcggttttaggcactccgattaccggtccgtggaaggaaggtcaacgctccctattagtagcgctgggatgtttctggggtcatgaaaaaatgtactgggagacagatggggtggaatctacatcggtaggctatgccggcggtaccacccccaacccgacttattttgaggtctgccgtggccaaaccaatcacgctgaggtcgtagaaattacctatgacccggaaaagattagcctgaaggaactcgtggtgatggcgcttgaagcccacgacccaacccagggctttaggcaaggtaatgacgtgggcacccagtaccgttccgcgttttatccacgtactcaggaagaactggaaatcatccaggaactggtggatagctatgacaagaagctcgccgaaaacggctttggcgccatgaccactgaggtcaaactgctcagtgacactgactctggcgagtactacctagcagaagacgagcaccagcaatacctctacaaggtgcctaatggctactgcccacaccactccaccggcgtgaagtgcgattag

SEQ ID NO: 3 - protein, 216 aa, Artificial Sequence
  WT AA
MSFLFAPTPQLVAKEDALPGRAEPILEPKPHAVLGTPITGPWKEGQRSLLVALGCFWGHEKMYWETDGVESTSVGYAGGTTPNPTYFEVCRGQTNHAEVVEITYDPEKISLKELVVMALEAHDPTQGFRQGNDVGTQYRSAFYPRTQEELEIIQELVDSYDKKLAENGFGAMTTEVKLLSDTDSGEYYLAEDEHQQYLYKVPNGYCPHHSTGVKCD

SEQ ID NO: 4 - DNA, 651 bp, Artificial Sequence
  WT NT
atgtcgttcttatttgcacctacccctcaacttgttgctaaagaagatgcattacccggccgcgcagaacctatcttggagcctaagccgcatgcggttttaggcactccgattaccggtccgtggaaggaaggtcaacgctccctattagtagcgctgggatgtttctggggtcatgaaaaaatgtactgggagacagatggggtggaatctacatcggtaggctatgccggcggtaccacccccaacccgacttattttgaggtctgccgtggccaaaccaatcacgctgaggtcgtagaaattacctatgacccggaaaagattagcctgaaggaactcgtggtgatggcgcttgaagcccacgacccaacccagggctttaggcaaggtaatgacgtgggcacccagtaccgttccgcgttttatccacgtactcaggaagaactggaaatcatccaggaactggtggatagctatgacaagaagctcgccgaaaacggctttggcgccatgaccactgaggtcaaactgctcagtgacactgactctggcgagtactacctagcagaagacgagcaccagcaatacctctacaaggtgcctaatggctactgcccacaccactccaccggcgtgaagtgcgattag

SEQ ID NO: 5 - DNA, 5803 bp, Artificial Sequence
  pDCM2
gttcgcttgctgtccataaaaccgcccagtctagctatcgccatgtaagcccactgcaagctacctgctttctctttgcgcttgcgttttcccttgtccagatagcccagtagctgacattcatccggggtcagcaccgtttctgcggactggctttctacgtgttccgcttcctttagcagcccttgcgccctgagtgcttgcggcagcgtgaagctagcttttatcgccattcgccattcaggctgcgcaactgttgggaagggcgatcggtgcgggcctcttcgctattacgccagctggcgaaagggggatgtgctgcaaggcgattaagttgggtaacgccagggttttcccagtcacgacgttgtaaaacgacggccagtgaattcgagctcggtacccggggatcctctagagtcgacctgcaggcatgcaagcttggcgtaatcatggtcatagctgtttcctgtgtgaaattgttatccgctcacaattccacacaacatacgagccggaagcataaagtgtaaagcctggggtgcctaatgagtgagctaactcacattaattgcgttgcgctcactgcccgctttccagtcgggaaacctgtcgtgccagctgcattaatgaatcggccaacgcgcggggagaggcggtttgcgtattgggcgctcttccgcttcctcgctcactgactcgctgcgctcggtcgttcggctgcggcgagcggtatcagctcactcaaaggcggtaatacggttatccacagaatcaggggataacgcaggaaagaacatgtgagcaaaaggccagcaaaaggccaggaaccgtaaaaaggccgcgttgctggcgtttttccataggctccgcccccctgacgagcatcacaaaaatcgacgctcaagtcagaggtggcgaaacccgacaggactataaagataccaggcgtttccccctggaagctccctcgtgcgctctcctgttccgaccctgccgcttaccggatacctgtccgcctttctcccttcgggaagcgtggcgctttctcaatgctcacgctgtaggtatctcagttcggtgtaggtcgttcgctccaagctgggctgtgtgcacgaaccccccgttcagcccgaccgctgcgccttatccggtaactatcgtcttgagtccaacccggtaagacacgacttatcgccactggcagcagccactggtaacaggattagcagagcgaggtatgtaggcggtgctacagagttcttgaagtggtggcctaactacggctacactagaaggacagtatttggtatctgcgctctgctgaagccagttaccttcggaaaaagagttggtagctcttgatccggcaaacaaaccaccgctggtagcggtggtttttttgtttgcaagcagcagattacgcgcagaaaaaaaggatctcaagaagatcctttgatcttttctacggggtctgacgctcagtggaacgaaaactcacgttaagggattttggtcatgagattatcaaaaaggatcttcacctagatccttttggggtgggcgaagaactccagcatgagatccccgcgctggaggatcatccagccctgatagaaacagaagccactggagcacctcaaaaacaccatcatacactaaatcagtaagttggcagcatcacccgacgcactttgcgccgaataaatacctgtgacggaagatcacttcgcagaataaataaatcctggtgtccctgttgataccgggaagccctgggccaacttttggcgaaaatgagacgttgatcggcacgtaagaggttccaactttcaccataatgaaataagatcactaccgggcgtattttttgagttatcgagattttcaggagctgatagaaacagaagccactggagcacctcaaaaacaccatcatacactaaatcagtaagttggcagcatcacccgacgcactttgcgccgaataaatacctgtgacggaagatcacttcgcagaataaataaatcctggtgtccctgttgataccgggaagccctgggccaacttttggcgaaaatgagacgttgatcggcacgtaagaggttccaactttcaccataatgaaataagatcactaccgggcgtattttttgagttatcgagattttcaggagctctttggcatcgtctctcgcctgtcccctcagttcagtaatttcctgcatttgcctgtttccagtcggtagatattccacaaaacagcagggaagcagcgcttttccgctgcataaccctgcttcggggtcattatagcgattttttcggtatatccatcctttttcgcacgatatacaggattttgccaaagggttcgtgtagactttccttggtgtatccaacggcgtcagccgggcaggataggtgaagtaggcccacccgcgagcgggtgttccttcttcactgtcccttattcgcacctggcggtgctcaacgggaatcctgctctgcgaggctggccggctaccgccggcgtaacagatgagggcaagcggatggctgatgaaaccaagccaaccaggaagggcagcccacctatcaaggtgtactgccttccagacgaacgaagagcgattgaggaaaaggcggcggcggccggcatgagcctgtcggcctacctgctggccgtcggccagggctacaaaatcacgggcgtcgtggactatgagcacgtccgcgagggcgtcccggaaaacgattccgaagcccaacctttcatagaaggcggcggtggaatcgaaatctcgtgatggcaggttgggcgtcgcttggtcggtcatttcgaaaaaggttaggaatacggttagccatttgcctgcttttatatagttcantatgggattcacctttatgttgataagaaataaaagaaaatgccaataggatatcggcattttcttttgcgtttttatttgttaactgttaattgtccttgttcaaggatgctgtctttgacaacagatgttttcttgcctttgatgttcagcaggaagctcggcgcaaacgttgattgtttgtctgcgtagaatcctctgtttgtcatatagcttgtaatcacgacattgtttcctttcgcttgaggtacagcgaagtgtgagtaagtaaaggttacatcgttaggcggatcaagatccatttttaacacaaggccagttttgttcagcggcttgtatgggccagttaaagaattagaaacataaccaagcatgtaaatatcgttagacgtaatgccgtcaatcgtcatttttgatccgcgggagtcagtgaacaggtaccatttgccgttcattttaaagacgttcgcgcgttcaatttcatctgttactgtgttagatgcaatcagcggtttcatcacttttttcagtgtgtaatcatcgtttagctcaatcataccgagagcgccgtttgctaactcagccgtgcgttttttatcgctttgcagaagtttttgactttcttgacggaagaatgatgtgcttttgccatagtatgctttgttaaataaagattcttcgccttggtagccatcttcagttccagtgtttgcttcaaatactaagtatttgtggcctttatcttctacgtagtgaggatctctcagcgtatggttgtcgcctgagctgtagttgccttcatcgatgaactgctgtacattttgatacgtttttccgtcaccgtcaaagattgatttataatcctctacaccgttgatgttcaaagagctgtctgatgctgatacgttaacttgtgcagttgtcagtgtttgtttgccgtaatgtttaccggagaaatcagtgtagaataaacggatttttccgtcagatgtaaatgtggctgaacctgaccattcttgtgtttggtcttttaggatagaatcatttgcatcgaatttgtcgctgtctttaaagacgcggccagcgtttttccagctgtcaatagaagtttcgccgactttttgatagaacatgtaaatcgatgtgtcatccgcatttttaggatctccggctaatgcaaagacgatgtggtagccgtgatagtttgcgacagtgccgtcagcgttttgtaatggccagctgtcccaaacgtccaggccttttgcagaagagatatttttaattgtggacgaatcaaattcagaaacttgatatttttcatttttttgctgttcagggatttgcagcatatcatggcgtgtaatatgggaaatgccgtatgtttccttatatggcttttggttcgtttctttcgcaaacgcttgagttgcgcctcctgccagcagtgcggtagtaaaggttaatactgttgcttgttttgcaaactttttgatgttcatcgttcatgtctccttttttatgtactgtgttagcggtctgcttcttccagccctcctgtttgaagatggcaagttagttacgcacaataaaaaaagacctaaaatatgtaaggggtgacgccaaagtatacactttgccctttacacattttaggtcttgcctgctttatcagtaacaaacccgcgcgatttacttttcgacctcattctattagactctcgtttggattgcaactggtctattttcctcttttgtttgatagaaaatcataaaaggatttgcagactacgggcctaaagaactaaaaaatctatctgtttcttttcattctctgtattttttatagtttctgttgcatgggcataaagttgcctttttaatcacaattcagaaaatatcataatatctcatttcactaaataatagtgaacggcaggtatatgtgatgggttaaaaaggatcaccccagagtcccgctcagaagaactcgtcaagaaggcgatagaaggcgatgcgctgcgaatcgggagcggcgataccgtaaagcacgaggaagcggtcagcccattcgccgccaagctcttcagcaatatcacgggtagccaacgctatgtcctgatagcggtccgccacacccagccggccacagtcgatgaatccagaaaagcggccattttccaccatgatattcggcaagcaggcatcgccatgggtcacgacgagatcctcgccgtcgggcatccgcgccttgagcctggcgaacagttcggctggcgcgagcccctgatgctcttcgtccagatcatcctgatcgacaagaccggcttccatccgagtacgtgctcgctcgatgcgatgtttcgcttggtggtcgaatgggcaggtagccggatcaagcgtatgcagccgccgcattgcatcagccatgatggatactttctcggcaggagcaaggtgagatgacaggagatcctgccccggcacttcgcccaatagcagccagtcccttcccgcttcagtgacaacgtcgagacagctgcgcaaggaacgcccgtcgtggccagccacgatagccgcgctgcctcgtcttggagttcattcagggcaccggacaggtcggtcttgacaaaaagaaccgggcgcccctgcgctgacagccggaacacggcggcatcagagcagccgattgtctgttgtgcccagtcatagccgaatagcctctccacccaagcggccggagaacctgcgtgcaatccatcttgttcaatcatgcgaaacgatcctcatcctgtctcttgatcagatcttgatcccctgcgccatcagatccttggcggcaagaaagccatccagtttactttgcagggcttcccaaccttaccagagggcgccccagctggcaattccg

SEQ ID NO: 6 - DNA, 35 bp, Artificial Sequence
  1F
tcgagctcggtacccagagaagtgagccttgaact

SEQ ID NO: 7 - DNA, 30 bp, Artificial Sequence
  2R
agttgaggggtaggtacaaataagaacgac

SEQ ID NO: 8 - DNA, 30 bp, Artificial Sequence
  3F
gtcgttcttatttgtacctacccctcaact

SEQ ID NO: 9 - DNA, 35 bp, Artificial Sequence
  4R
ctctagaggatcccctgtcatagctatccaccagt

SEQ ID NO: 10 - DNA, 20 bp, Artificial Sequence
  5F
agagaagtgagccttgaact

SEQ ID NO: 11 - DNA, 20 bp, Artificial Sequence
  6R
tgtcatagctatccaccagt